European Patent Application EP 4 722 702 A1, published April 8, 2026. Title: Modification analysis of molecule by signal-based method. Applicant: The University of Tokyo. Application JP. The sequence listing filed with the application follows.

SEQUENCE LISTING (7 sequences)

SEQ ID NO: 1 - DNA, 10 bp, synthetic construct
  source 1..10: mol_type = other DNA
  misc_feature 1..10: note = part of 3 adapter
tagtaggttc

SEQ ID NO: 2 - RNA, 14 nt, synthetic construct
  source 1..14: mol_type = other RNA
  misc_feature 1..14: note = 5 adapter A
gggaggatactgga

SEQ ID NO: 3 - RNA, 14 nt, synthetic construct
  source 1..14: mol_type = other RNA
  misc_feature 1..14: note = 5 adapter U
gggaggatactggt

SEQ ID NO: 4 - RNA, 14 nt, synthetic construct
  source 1..14: mol_type = other RNA
  misc_feature 1..14: note = 5 adapter C
gggaggatactggc

SEQ ID NO: 5 - RNA, 14 nt, synthetic construct
  source 1..14: mol_type = other RNA
  misc_feature 1..14: note = 5 adapter G
gggaggatactggg

SEQ ID NO: 6 - RNA, 13 nt, synthetic construct
  source 1..13: mol_type = other RNA
  misc_feature 1..13: note = 5 adapter for His
gggaggatactgg

SEQ ID NO: 7 - DNA, 50 bp, synthetic construct
  misc_feature 41..50: note = DNA
  misc_feature 1..40: note = RNA
  source 1..50: mol_type = other DNA
  misc_feature 1..50: note = 3 adapter
gtatcctcccagagagagagagagagagagagattccccctagtaggttc